European Patent Specification EP 3 762 725 B1, published October 23, 2024. Title: SPECIES SPECIFIC ANTIGEN SEQUENCES FOR TICK-BORNE RELAPSING FEVER (TBRF) AND METHODS OF USE. Applicant: ID-FISH TECHNOLOGIES, INC. Application TBD. The sequence listing filed with the application follows.

SEQUENCE LISTING (20 sequences)

SEQ ID NO: 1 - protein, 259 aa, Borrelia hermsii
MSESNWEIDEPGSVQDIRNSVASELQKPENIGQRGKSVGKEVGKDAAASGEGAVVAVGSKQNTLQNSENSSQEGAGSALQKPGDSPQKGVASQEGTNGALQGVVAAGGVSVGGSGVGAAASDGNSSSSQEAESVDLKNVLADSHGVGASNLNIKAEGDISTGHGTEGVIASGDLTNTIITSGVTAAASPAIVSGDERGVAAIKDSIAVVLETQKEAQKETEKETENVKFAVLGTVKKIVDGVADGIANVIEYGLENGID

SEQ ID NO: 2 - protein, 257 aa, Borrelia hermsii
MNKVKDGIKTASKGAETFVTAAMQGAGAVLGSLQDVGNFVMDATLSMGDMFAGIKSDSDVSSANSGMTVNSGMTVSLSSNETQVIGHLEEYLKSAIKVNGNESSRQSKLENGRQKFFAWLREKDTDFSKRKELVQAMQRVYNFIKEKSSNSRELQTWVLGVVGDDDTVVDVDRDDELNSDVEIDFLIKKTLSSRDYSGFAVSLLFQALADTLYDAENDRDKPEEQIFKDLKAVFSDNAGEDKGFGEFKSIIEDKSQA

SEQ ID NO: 3 - protein, 260 aa, Borrelia miyamotoi
MAKAGNFDEVLDLDGDDEEAEIDEIEQNLSEGVDGNIDQNPGNVDGHIVLVDAQGVSVPTVVEHSAVSSSVERRVVTVGQNVESRRLTKVERLEKYLESAIKSGGKLNEQQRRLKNGKQMLFTWLNEDANASKRAELEQDMQKLYGLIKESITDSSSQFSSRDGEYSDEAIDGLLNSLFSSSFDNTFALDLFFQALLNTLCDFKKDNCKDEEVIFADIRKVFSDESDTKGHFGYLKSKLKDELVISDEGDYGEDEDFEED

SEQ ID NO: 4 - protein, 224 aa, Borrelia turcica
MEEEASIESEAMPLDEAKISSLDKETVPAVQADGTPEQIVASVGLEGEESKKFEHLKGSLGDAIKVNGKGEEKRKENEERQKEFFDWLDKNDPDLSKRKELAELMKKVYGLLKEHAQNSEQIKSFVEGTPKDENVKKIGVTSARDIKTDEQVEALIKAVLGHSEESGTNLSLFFQKLGDAFGTEDGESQKSNEKILEELKRVCESSDEIKKLKEDLKIEEKVQS

SEQ ID NO: 5 - protein, 226 aa, Borrelia turcica
MNIDAVADLLADQQEAASTGLKDASTGLKDTSTGLSKLDKKEKKVSSLKETLENSSNVLYESSSPTKTRQEEFFKWLEENDSDYSKRKQLEESMDKVFSLIKDSASSSTEIKEIIAKGQSDAGIIKAGIKTADDIKTDEQVDALVKFVTGTGDDLDLESGSSSIKAFFGTLAEVFDDDLNDVMTDKKGQKRGHDKVFEDLKKVFSEDSDGPFDILKDALKQALKNN

SEQ ID NO: 6 - protein, 250 aa, Borrelia turicatae
MSTSYWSVDNDGFVQGTKSFVDSPLRKPDRFDQEVSAGGKKIEKAVSRNLRVAGGQRQGIADDGIGVAGVREAGGVLKDAGNAVQRDINGSGEGIKNDVIQNPEGVGVQVAVGSADTGADSGQEAGKVFQNLGDTGTQSIQRVVSSSDLNSDLGVGSKDGISTNGMSTNHVTENENSINSITSTSSGLNTALQMAGTSTRTSGYEGEITTNTQDRTFVETGTQDSKAQYSDFSDQDIRDKVLGSVVGGVV

SEQ ID NO: 7 - protein, 334 aa, Borrelia hermsii
MASMTGGQQMGRGSEKMSQNQKSPLVIAHRGASGYLPEHTLEAKAYAYALGADYLEQDIVLTKDNIPVIMHDPELDTTTNVAKLFPERARENGRYYSVDFTLDELKSLSLSERFDPASRNPIYPNRFPLNEHDFKIPTLEEEIQFIQGLNKSTGRNVGIYPEIKKPLWHKQQGKDISKIVIEILNKYGYKSKEDKIYLQTFDFDELKRIREELGYQGKLIMLVGENDWDEAPTDYEYIKSEEGMAEVAKYSDGIGPWIPQIIIEGKITDLTSLAHKHNMEVHPYTFRIDALPSYVKDADELLDLLFNKAKVDGIFTDFTDTVVNFITKIKPKGE

SEQ ID NO: 8 - protein, 254 aa, Borrelia miyamotoi
MASMTGGQQMGRGSEMGENKKSPLIIAHRGASGYLPEHTLEAKAYAYALGADYLEQDIVLTKDNIPVIMHDPEIDTTTNVAQLFPNRARENGRYYATDFTLTELKSLNLSERFDPENKKPIYPNRFPLNEYNFKIPTLEEEIQFIQGLNKSTGKNVGIYPEIKKPFWHKQQGKDISKIVIEILNKYGYKSKEDKIYLQTFDFDELKRIRKELGYQGKLIMLVGENDWNEAPTDYEYIKSEEGIAEVAKYSDGIG

SEQ ID NO: 9 - protein, 327 aa, Borrelia turcica
MASMTGGQQMGRGSKVSMNKALPLVIAHRGASGYLPEHTLEAKAFAYALGAHYLEQDIVLTKDDIPIIMHDPEIDTTTNVAEIFPERARKDGRYYSVDFTLRELKSLKLSERFDPKTGKPIYPNRFPLNEYNFKIPTLEEEIQFIQGLNKSTGRNVGIYPEIKKPFWHKQQGKDISKIVIEMLNKYGYKSKEDKIYLQIFDFDELKRIREELGYKGKLVMLIGENDWNEAPTDYEYIKSEEGIAEVAKYSDGIGPWIPQVIIDGKVTGLTSLAHKHKMEVHPYTMRIDALPSYVKDANELLNLLFNKAKVDGVFTDFPDVVLGFIRK

SEQ ID NO: 10 - protein, 329 aa, Borrelia turicatae
MASMTGGQQMGRGSEKMSMTNKKPPLIIAHRGASGYLPEHTLEAKAFAYALGADYLEQDIVLTKDNVPIIMHDPELDTTTNVAKLFPERARENGRYYSVDFTLDELKSLSLSERFDLETRKPIYPNRFPLNEYNVKIPTLEEEIQFIQGLNKSTGRNVGIYPEIKKPLWHKQQGKDISKIVIEILNKYGYKSKEDKIYLQTFDFDELKRIREELGYQGKLIMLVGENDWDEAPTDYEYIKSQEGMTEVAKYADGIGPWIPQIIIDGKITDLTSLAHKYNMEVHAYTFRIDSLPSYVKDANELLDLLFNKAKIDGLFTDFTDTVVKFVKQ

SEQ ID NO: 11 - protein, 171 aa, Borrelia hermsii
MASMTGGQQMGRGSSDANLLKTLDNNQKQALIYFKDTLQDKKYLNDLTASQKNFLDDLEKNKKDPGLQDKLKKTLSSEYDGSQFNKLLNELGNAKVKQFLQQLHIMLQSIKDGTLTSFSYANFKDLQTLEQKKERALQYINGRLYVEYYFYINGISNADNFFESVMQLLET

SEQ ID NO: 12 - protein, 169 aa, Borrelia miyamotoi
MLDHNLQPNKINNIISSLDSNQKQALIFFKNLVKNKQYSKDLEQASKSYLENLKEKNNQNLNLQNKLNQGLNCDYDDSKIEKLFDQLGNDKMKKFLQQLHLMLKSINDGTLISFSSSNFRDTTTLSQKKEKALEYIKSQLYIEFYFHSNDISDTEFFFQRTIALLETQN

SEQ ID NO: 13 - protein, 322 aa, Borrelia hermsii
MRNNSINATNLSKTQEKLSSGHRINRASDDAAGMGVAGKINAQIRGLSQASRNTSKAINFIQTTEGNLNEVERVLVRMKELAVQSGNGTYSDADRGSIQIEIEQLTDEINRIADQAQYNQMHMLSNKSAAQNVKTAEELGMQPAKINTPASLAGSQASWTLRVHVGANQDEAIAVNIYASNVANLFAGEGAQAAPVQEIGQQEEGQAAPAPAAAPAQGGVNSPINVTTAVDANMSLAKIEGAIRMVSDQRANLGAFQNRLESIKDSTEYAIENLKASYAQIKDATMTDEVVASTTHSILTQSAMAMIAQANQVPQYVLSLLR

SEQ ID NO: 14 - protein, 322 aa, Borrelia miyamotoi
MRNNGINAANLSKTQEKLSSGYRINRASDDAAGMGVAGKLNSQIRGLSQASRNTSKAINFIQTTEGNLNEVEKVLVRMKELAVQSGNGTYSDSDRGSIQIEIEQLTDEINRIADQAQYNQMHMLSNKSAAQNVKTAEELGMQPAKINTPASLAGSQASWTLRVHVGANQDEAIAVNIYAANVANLFNGEGAQAAPAQEGAQQEGVQAVPAPAAAPVQGGVNSPINVTTAIDANMSLSKIEDAIRMVTDQRANLGAFQNRLESVKASTDYAIENLKASYAQVKDAIMTDEIVASTTNSILTQSAMAMIAQANQVPQYVLSLLR

SEQ ID NO: 15 - protein, 324 aa, Borrelia turcica
MRNNGINASNLSKTQEKLSSGYRINRASDDAAGMGVAGKINAQIRGLSQASRNTSKAINFIQTTEGNLNEVEKVLVRMKELAVQSGNGTYSDADRGSIQIEIEQLTDEINRIADQSQYNQMHMLSNKSAAQNVKTAEELGMQPAKINTPASLSGAQASWTLRVHVGANQDEAIAVNIYAANVPNLFAGEGAQTAAAAPAQAGTQQEGAQEPAAAAAPAQGGVNSPVNVTTTVDANMSLAKIENAIRMISDQRANLGAFQNRLESIKNSTEYSIENLKASYAQIKDATMTDEIVSSTTNSILTQSAMAMIAQANQVPQYVLSLLR

SEQ ID NO: 16 - protein, 320 aa, Borrelia hermsii
MSKAGSGLTKIAILVDGTFDDESFNGSAWKGAKKVEKEFGLEIMMKESNANSYLADLESLKNNGSNFLWLIGYKFSDFAIIAALENPESKYVIIDPVYESDLVIPENLSAITFRTEEGAFLVGYIAAKMSKTGKIGFLGGFDDVVVNTFRYGYEAGAIYANKHINIDNKYIGNFVNTETGKNMANAMYAEGVDIIYHVAGLAGLGVIESARDLGDGHYVIGVDQDQSHLAPDNVITSSIKDIGRVLNIMISNYLKTNAFEGGQVLSYGLKEGFLDFVKNPKMISFELEKELDDLSEGIINGKIIVPNNERTYNQFMRKIL

SEQ ID NO: 17 - protein, 202 aa, Borrelia hermsii
MFLFISCNNGGPELKGNEVAKSDGTVLDLSKISTKIKNAGAFAASVQEVATLVKSVDELASAIGKKIKEDGTLDTLNNKNGSLLAGAFQVILTVEAKLKELEKQDGLSVELRAKVTSAKSASSGLVNKLKGGHAELGIEGATDENAQKAIKKDNGDQSKGAEELGKLNTAIGALLSAANDAVEAAIKELTAAPAKPATPAKP

SEQ ID NO: 18 - protein, 337 aa, Borrelia coriaceae
MKSMKPKLLMLIINIFLIISCQNEKVSMNEKSPLIIAHRGASGYLPEHTLEAKAYAYALGADYLEQDIVLTKDNVPIIMHDSELDTTTNVAKLFPERARENGKYYAVDFTLDEIKSLSISERFDPETREPIYPNRFPLNEYNFKIPTLEEEIQFIQGLNKSTGKNVGIYPEIKKPFWHKQQGKDISKIVIEILNQYGYKSKEDKIYLQTFDFDELKRIREELGYQGKLIMLVGENDWNEAPTDYEYIKSQEGMTEVAKYADGIGPWISQIIIDGQVTDLISLAHKHNMEVHPYTFRIDALPSYVKDANELLDLLFNKAQVDGIFTDFVDKAMEFVKK

SEQ ID NO: 19 - protein, 562 aa, Borrelia coriaceae
MKSFSVFILFLSTFTLSCKFYDTANASDLQADGDKFSQGFSSFNDILPFSDLKINKDVSTGSLKAQGTSSIKGDEKKGKGTSKDPIKDQEASGLKGVGVAGAGAKSFGDDGKKEEVVSKDSLKNEGTSGTAEVLKVSKEVEVAGVDTAKPAGGNGEEVASISENYLQNQETLVAQGAGVGSVGDAIGDRSLFFKNTDSNNAEQVVATEDLLVGASEGVNTSDLGLKVAIPTDHVRGDVVATETQNAEKKGDKTQNTELASLDIKDNITVNVVDGTKININKNSSNTNESINVTKDGVNTVIKGVETSIKTADGKVVVKKRTLKKGLKKKNSKKQASKSKTPEAAVVGNKKNVDTNMSSVIGLDSEALGKDKNIDLDSKSDETYVIERVEKLAKYLQSAIKINGKKVEEQDKLEAGRQKFFEWLSKNDTDLLKRKALVQDLQKIYDLMKDKIADSTELQDWFQIVSDDIGDEETNIIDVESYYELSSDTEIDFLLERTLEDENYSGFSISLFMQALADTLYDIQNDSHKSGEEILQELKRVFDDTFYKIRGFEEFKSQIAAED

SEQ ID NO: 20 - protein, 193 aa, Borrelia coriaceae
MKLTKKYLLAVLLLSLINCDLLSKNKILTSHLLNTLDNNKKEALVTFKNLLQDKSHLEYLKSEQAKMLTNFTEDDGIEQPHLQEKLKGTLSSEYNENQLNQLFSELGYEKTKQFLDNLHKMLQAIKDGTLRAFHDSSSFKDYNTTLEAKKAEALSSVKKELYVQYYFYINDLQTADDFFVLTRNHLMIFKNNL